European Patent Application EP 4 115 874 A1, published January 11, 2023. Title: DELIVERY OF MRNA FOR THE AUGMENTATION OF PROTEINS AND ENZYMES IN HUMAN GENETIC DISEASES. Applicant: SHIRE HUMAN GENETIC THERAPIES. Application PCT/US2010/058457. The sequence listing filed with the application follows.

SEQUENCE LISTING (3 sequences)

SEQ ID NO: 1 - RNA, 1672 nt, Artificial
  CO-FF Luciferase mRNA
gggauccuaccauggaagaugccaaaaacauuaagaagggcccagcgccauucuacccacucgaagacgggaccgccggcgagcagcugcacaaagccaugaagcgcuacgcccuggugcccggcaccaucgccuuuaccgacgcacauaucgagguggacauuaccuacgccgaguacuucgagaugagcguucggcuggcagaagcuaugaagcgcuaugggcugaauacaaaccaucggaucguggugugcagcgagaauagcuugcaguucuucaugcccguguugggugcccuguucaucgguguggcuguggccccagcuaacgacaucuacaacgagcgcgagcugcugaacagcaugggcaucagccagcccaccgucguauucgugagcaagaaagggcugcaaaagauccucaacgugcaaaagaagcuaccgaucauacaaaagaucaucaucauggauagcaagaccgacuaccagggcuuccaaagcauguacaccuucgugacuucccauuugccacccggcuucaacgaguacgacuucgugcccgagagcuucgaccgggacaaaaccaucgcccugaucaugaacaguaguggcaguaccggauugcccaagggcguagcccuaccgcaccgcaccgcuuguguccgauucagucaugcccgcgaccccaucuucggcaaccagaucauccccgacaccgcuauccucagcguggugccauuucaccacggcuucggcauguucaccacgcugggcuacuugaucugcggcuuucgggucgugcucauguaccgcuucgaggaggagcuauucuugcgcagcuugcaagacuauaagauucaaucugcccugcuggugcccacacuauuuagcuucuucgcuaagagcacucucaucgacaaguacgaccuaagcaacuugcacgagaucgccagcggcggggcgccgcucagcaaggagguaggugaggccguggccaaacgcuuccaccuaccaggcauccgccagggcuacggccugacagaaacaaccagcgccauucugaucacccccgaaggggacgacaagccuggcgcaguaggcaagguggugcccuucuucgaggcuaaggugguggacuuggacaccgguaagacacugggugugaaccagcgcggcgagcugugcguccguggccccaugaucaugagcggcuacguuaacaaccccgaggcuacaaacgcucucaucgacaaggacggcuggcugcacagcggcgacaucgccuacugggacgaggacgagcacuucuucaucguggaccggcugaagagccugaucaaauacaagggcuaccagguagccccagccgaacuggagagcauccugcugcaacaccccaacaucuucgacgccggggucgccggccugcccgacgacgaugccggcgagcugcccgccgcagucgucgugcuggaacacgguaaaaccaugaccgagaaggagaucguggacuauguggccagccagguuacaaccgccaagaagcugcgcggugguguuguguucguggacgaggugccuaaaggacugaccggcaaguuggacgcccgcaagauccgcgagauucucauuaaggccaagaagggcggcaagaucgccguguaauuugaauu

SEQ ID NO: 2 - RNA, 157 nt, Artificial
  5' CMV Sequence
uaauacgacucacuauaggacagaucgccuggagacgccauccacgcuguuuugaccuccauagaagacaccgggaccgauccagccuccgcggccgggaacggugcauuggaacgcggauuccccgugccaagagugacucaccguccuugacacg

SEQ ID NO: 3 - RNA, 100 nt, Artificial
  3' hGH Sequence
cggguggcaucccugugaccccuccccagugccucuccuggcccuggaaguugccacuccagugcccaccagccuuguccuaauaaaauuaaguugcauc